European Patent Application EP 4 588 942 A1, published July 23, 2025. Title: Truncated respiratory syncytial virus F protein and use thereof. Applicant: XIAMEN UNIVERSITY. Application CN. The sequence listing filed with the application follows.

SEQUENCE LISTING (46 sequences)

SEQ ID NO: 1 - protein, 574 aa, synthetic construct
MELLILKANAITTILTAVTFCFASGQNITEEFYQSTCSAVSKGYLSALRTGWYTSVITIELSNIKKNKCNGTDAKVKLIKQELDKYKNAVTELQLLMQSTQATNNRARRELPRFMNYTLNNAKKTNVTLSKKRKRRFLGFLLGVGSAIASGVAVSKVLHLEGEVNKIKSALLSTNKAVVSLSNGVSVLTSKVLDLKNYIDKQLLPIVNKQSCSISNIETVIEFQQKNNRLLEITREFSVNAGVTTPVSTYMLTNSELLSLINDMPITNDQKKLMSNNVQIVRQQSYSIMSIIKEEVLAYVVQLPLYGVIDTPCWKLHTSPLCTTNTKEGSNICLTRTDRGWYCDNAGSVSFFPQAETCKVQSNRVFCDTMNSLTLPSEVNLCNVDIFNPKYDCKIMTSKTDVSSSVITSLGAIVSCYGKTKCTASNKNRGIIKTFSNGCDYVSNKGVDTVSVGNTLYYVNKQEGKSLYVKGEPIINFYDPLVFPSDEFDASISQVNEKINQSLAFIRKSDELLHNVNAGKSTTNIMITTIIIVIIVILLSLIAVGLLLYCKARSTPVTLSKDQLSGINNIAFSN

SEQ ID NO: 2 - protein, 6 aa, synthetic construct
GGGPGG

SEQ ID NO: 3 - protein, 251 aa, synthetic construct
SAVSKGYLSALRTGWYTSVITIELSNIKKIKCNGTDAKIKLIKQELDKYKNAVTELQLLMQSTPATNNGGGPGGSAIASGVAVSKVLHLEGEVNKIKSALLSTNKAVVSLSNGVSVLTSKVLDLKNYIDKQLLPIVNKQSCSIPNIETVIEFQQKNNRLLEITREFSVNAGVTTPVSTYMLTNSELLSLINDMPITNDQKKLMSNNVQIVRQQSYSIMSIIKEEVLAYVVQLPLYGVIDTPCWKLHTSPLC

SEQ ID NO: 4 - protein, 222 aa, synthetic construct
GWYTSVITIELSNIKENKCNGTDAKVKLIKQELDKYKNAVTELQLLMQSTPATNNGGGPGGSAIASGVAVSKVLHLEGEVNKIKSALLSTNKAVVSLSNGVSVLTSKVLDLKNYIDKQLLPIVNKQSCSISNIETVIEFQQKNNRLLEITREFSVNAGVTTPVSTYMLTNSELLSLINDMPITNDQKKLMSNNVQIVRQQSYSIMSIIKEEVLAYVVQLPLY

SEQ ID NO: 5 - protein, 217 aa, synthetic construct
VITIELSNIKENKCNGTDAKVKLIKQELDKYKNAVTELQLLMQSTPATNNGGGPGGSAIASGVAVSKVLHLEGEVNKIKSALLSTNKAVVSLSNGVSVLTSKVLDLKNYIDKQLLPIVNKQSCSISNIETVIEFQQKNNRLLEITREFSVNAGVTTPVSTYMLTNSELLSLINDMPITNDQKKLMSNNVQIVRQQSYSIMSIIKEEVLAYVVQLPLY

SEQ ID NO: 6 - protein, 213 aa, synthetic construct
GWYTSVITIELSNIKENKCNGTDAKVKLIKQELDKYKNAVTELQLLMQSTPATNNGGGPGGSAIASGVAVSKVLHLEGEVNKIKSALLSTNKAVVSLSNGVSVLTSKVLDLKNYIDKQLLPIVNKQSCSISNIETVIEFQQKNNRLLEITREFSVNAGVTTPVSTYMLTNSELLSLINDMPITNDQKKLMSNNVQIVRQQSYSIMSIIKEEVL

SEQ ID NO: 7 - protein, 209 aa, synthetic construct
VITIELSNIKENKCNGTDAKVKLIKQELDKYKNAVTELQLLMQSTPATNNGGGPGGSAIASGVAVSKVLHLEGEVNKIKSALLSTNKAVVSLSNGVSVLTSKVLDLKNYIDKQLLPIVNKQSCSISNIETVIEFQQKNNRLLEITREFSVNAGVTTPVSTYMLTNSELLSLINDMPITNDQKKLMSNNVQIVRQQSYSIMSIIKEEVLG

SEQ ID NO: 8 - protein, 26 aa, synthetic construct
IMITTIIIVIIVILLSLIAVGLLLYC

SEQ ID NO: 9 - protein, 22 aa, synthetic construct
MDAMKRGLCCVLLLCGAVFVSA

SEQ ID NO: 10 - protein, 546 aa, synthetic construct
ATMELLILKANAITTILTAVTFCFASGQNITEEFYQSTCSAVSKGYLSALRTGWYTSVITIELSNIKKIKCNGTDAKIKLIKQELDKYKNAVTELQLLMQSTPATNNQARGSGSGRSLGFLLGVGSAIASGVAVSKVLHLEGEVNKIKSALLSTNKAVVSLSNGVSVLTSKVLDLKNYIDKQLLPIVNKQSCSIPNIETVIEFQQKNNRLLEITREFSVNAGVTTPVSTYMLTNSELLSLINDMPITNDQKKLMSNNVQIVRQQSYSIMSIIKEEVLAYVVQLPLYGVIDTPCWKLHTSPLCTTNTKEGSNICLTRTDRGWYCDNAGSVSFFPQAETCKVQSNRVFCDTMNSLTLPSEVNLCNVDIFNPKYDCKIMTSKTDVSSSVITSLGAIVSCYGKTKCTASNKNRGIIKTFSNGCDYVSNKGVDTVSVGNTLYYVNKQEGKSLYVKGEPIINFYDPLVFPSDQFDASISQVNEKINQSLAFIRKSDELLSAIGGYIPEAPRDGQAYVRKDGEWVLLSTFLGGIEGRHHHHHHSAWSHPQFEK

SEQ ID NO: 11 - protein, 530 aa, synthetic construct
MELLILKANAITTILTAVTFCFASGQNITEEFYQSTCSAVSKGYLSALRTGWYTSVITIELSNIKENKCNGTDAKVKLIKQELDKYKNAVTELQLLMQSTPATNNRARRELPRFMNYTLNNAKKTNVTLSKKRKRRAIASGVAVSKVLHLEGEVNKIKSALLSTNKAVVSLSNGVSVLTSKVLDLKNYIDKQLLPIVNKQSCSISNIETVIEFQQKNNRLLEITREFSVNAGVTTPVSTYMLTNSELLSLINDMPITNDQKKLMSNNVQIVRQQSYSIMSIIKEEVLAYVVQLPLYGVIDTPCWKLHTSPLCTTNTKEGSNICLTRTDRGWYCDNAGSVSFFPQAETCKVQSNRVFCDTMNSLTLPSEVNLCNVDIFNPKYDCKIMTSKTDVSSSVITSLGAIVSCYGKTKCTASNKNRGIIKTFSNGCDYVSNKGVDTVSVGNTLYYVNKQEGKSLYVKGEPIINFYDPLVFPSDEFDASISQVNEKINQSLAFIRKSDELLGLEVLFQGPHHHHHHHHSAWSHPQFEK

SEQ ID NO: 12 - protein, 438 aa, synthetic construct
FLGFLLGVGSAIASGVAVSKVLHLEGEVNKIKSALLSTNKAVVSLSNGVSVLTSKVLDLKNYIDKQLLPIVNKQSCSISNIETVIEFQQKNNRLLEITREFSVNAGVTTPVSTYMLTNSELLSLINDMPITNDQKKLMSNNVQIVRQQSYSIMSIIKEEVLAYVVQLPLYGVIDTPCWKLHTSPLCTTNTKEGSNICLTRTDRGWYCDNAGSVSFFPQAETCKVQSNRVFCDTMNSLTLPSEVNLCNVDIFNPKYDCKIMTSKTDVSSSVITSLGAIVSCYGKTKCTASNKNRGIIKTFSNGCDYVSNKGVDTVSVGNTLYYVNKQEGKSLYVKGEPIINFYDPLVFPSDEFDASISQVNEKINQSLAFIRKSDELLHNVNAGKSTTNIMITTIIIVIIVILLSLIAVGLLLYCKARSTPVTLSKDQLSGINNIAFSN

SEQ ID NO: 13 - protein, 84 aa, synthetic construct
QNITEEFYQSTCSAVSKGYLSALRTGWYTSVITIELSNIKKNKCNGTDAKVKLIKQELDKYKNAVTELQLLMQSTQATNNRARR

SEQ ID NO: 14 - protein, 177 aa, synthetic construct
SAIASGVAVSKVLHLEGEVNKIKSALLSTNKAVVSLSNGVSVLTSKVLDLKNYIDKQLLPIVNKQSCSISNIETVIEFQQKNNRLLEITREFSVNAGVTTPVSTYMLTNSELLSLINDMPITNDQKKLMSNNVQIVRQQSYSIMSIIKEEVLAYVVQLPLYGVIDTPCWKLHTSPLC

SEQ ID NO: 15 - protein, 161 aa, synthetic construct
SAIASGVAVSKVLHLEGEVNKIKSALLSTNKAVVSLSNGVSVLTSKVLDLKNYIDKQLLPIVNKQSCSISNIETVIEFQQKNNRLLEITREFSVNAGVTTPVSTYMLTNSELLSLINDMPITNDQKKLMSNNVQIVRQQSYSIMSIIKEEVLAYVVQLPLY

SEQ ID NO: 16 - protein, 75 aa, synthetic construct
EFYQSTCSAVSKGYLSALRTGWYTSVITIELSNIKKNKCNGTDAKVKLIKQELDKYKNAVTELQLLMQSTQATNN

SEQ ID NO: 17 - protein, 55 aa, synthetic construct
GWYTSVITIELSNIKKNKCNGTDAKVKLIKQELDKYKNAVTELQLLMQSTQATNN

SEQ ID NO: 18 - protein, 6 aa, synthetic construct
GGGSGG

SEQ ID NO: 19 - protein, 313 aa, synthetic construct
MDAMKRGLCCVLLLCGAVFVSAGGGSGGSAVSKGYLSALRTGWYTSVITIELSNIKKIKCNGTDAKIKLIKQELDKYKNAVTELQLLMQSTPATNNGGGPGGSAIASGVAVSKVLHLEGEVNKIKSALLSTNKAVVSLSNGVSVLTSKVLDLKNYIDKQLLPIVNKQSCSIPNIETVIEFQQKNNRLLEITREFSVNAGVTTPVSTYMLTNSELLSLINDMPITNDQKKLMSNNVQIVRQQSYSIMSIIKEEVLAYVVQLPLYGVIDTPCWKLHTSPLCGGSGGSGGIMITTIIIVIIVILLSLIAVGLLLYC

SEQ ID NO: 20 - protein, 284 aa, synthetic construct
MDAMKRGLCCVLLLCGAVFVSAGGGSGGGWYTSVITIELSNIKENKCNGTDAKVKLIKQELDKYKNAVTELQLLMQSTPATNNGGGPGGSAIASGVAVSKVLHLEGEVNKIKSALLSTNKAVVSLSNGVSVLTSKVLDLKNYIDKQLLPIVNKQSCSISNIETVIEFQQKNNRLLEITREFSVNAGVTTPVSTYMLTNSELLSLINDMPITNDQKKLMSNNVQIVRQQSYSIMSIIKEEVLAYVVQLPLYGGSGGSGGIMITTIIIVIIVILLSLIAVGLLLYC

SEQ ID NO: 21 - protein, 29 aa, synthetic construct
GYIPEAPRDGQAYVRKDGEWVLLSTFLGS

SEQ ID NO: 22 - protein, 335 aa, synthetic construct
TTAPSVYPLAPVCGGTTGSSVTLGCLVKGYFPEPVTLTWNSGSLSSGVHTFPALLQSGLYTLSSSVTVTSNTWPSQTITCNVAHPASSTKVDKKIEPRVPITQNPCPPLKECPPCAAPDLLGGPSVFIFPPKIKDVLMISLSPMVTCVVVDVSEDDPDVQISWFVNNVEVHTAQTQTHREDYNSTLRVVSALPIQHQDWMSGKAFACAVNNRALPSPIEKTISKPRGPVRAPQVYVLPPPAEEMTKKEFSLTCMITGFLPAEIAVDWTSNGRTEQNYKNTATVLDSDGSYFMYSKLRVQKSTWERGSLFACSVVHEGLHNHLTTKTISRSLGKGG

SEQ ID NO: 23 - protein, 6 aa, synthetic construct
GGGSGP

SEQ ID NO: 24 - protein, 4 aa, synthetic construct
GGSG

SEQ ID NO: 25 - protein, 10 aa, synthetic construct
GGGSGGGSPG

SEQ ID NO: 26 - protein, 5 aa, synthetic construct
EAAAK

SEQ ID NO: 27 - protein, 4 aa, synthetic construct
PAAK

SEQ ID NO: 28 - protein, 222 aa, synthetic construct
GWYTSVITIELSNIKENKCNGTDAKVKLLKQELDKYKNAVTELQLLMQSTPATNNGGGPGGSAIASGVAVSKVLHLEGEVNKIKSALLSTNKAVVSLSNGVSVLTSKVLDLKNYIDKQLLPIVNKQSCSISNIETVIEFQQKNNRLLEITREFSVNAGVTTPVSTYMLTNSELLSLINDMPITNDQKKLMSNNVQIVRQQSYSIMSIIKEEMLAYVVQLPLY

SEQ ID NO: 29 - protein, 222 aa, synthetic construct
GWYTSVITIELSNIKENKCNGTDAKVKLLKQELDKYKNAVTELQLLMQSTPATNNGGGPGGSAIASGVAVSKVLHLEGEVNKIKSALLSTNKAVVSLSNGVSVLTSKVLDLKNYIDKQLLPIVNKQSCSISNIETVIEFQQKNNRLLEITREFSVNAGVTTPVSTYMLTNSELLSLINDMPITNDQKKLMSNNVQIVRQQSYSIMSIIKEEVLLYVVQLPLY

SEQ ID NO: 30 - protein, 222 aa, synthetic construct
GWYTSVITIELSNIKENKCNGTDAKVKLLKQELDKYKNAVTELQLLMQSTPATNNGGGPGGSAIASGVAVSKVLHLEGEVNKIKSALLSTNKAIVSLSNGVSVLTSKVLDLKNYIDKQLLPIVNKQSCSISNIETVIEFQQKNNRLLEITREFSVNAGVTTPVSTYMLTNSELLSLINDMPITNDQKKLMSNNVQIVRQQSYSIMSIIKEEVLAYVVQLPLY

SEQ ID NO: 31 - protein, 222 aa, synthetic construct
GWYTSVITIELSNIKENKCNGTDAKVKLIKQELDKYKNAVTELQLLAQSTPATNNGGGPGGSAIASGVAVSKVLHLEGEVNKIKSALLSTNKAVVSLSNGVSVLTSKVLDLKNIIDKQLLPIVNKQSCSISNIETVIEFQQKNNRLLEITREFSVNAGVTTPVSTYMLTNSELLSLINDMPITNDQKKLMSNNVQIVRQQSYSIMSIIKEEVLAYVVQLPLY

SEQ ID NO: 32 - protein, 222 aa, synthetic construct
GWYTSVITIELSNIKENKCNGTDAKVKLLKQELDKYKNAVTELQLLAQSTPATNNGGGPGGSAIASGVAVSKVLHLEGEVNKIKSALLSTNKAVVSLSNGISVLTSKVLDLKNYIDKQLLPIVNKQSCSISNIETVIEFQQKNNRLLEITREFSVNAGVTTPVSTYMLTNSELLSLINDMPITNDQKKLMSNNVQIVRQQSYSIMSIIKEEVLLYVVQLPLY

SEQ ID NO: 33 - protein, 222 aa, synthetic construct
GWYTSVITIELSNIKENKCNGTDAKVKLIKQELDKYKNAVTELQLLMQSTPATNNGGGPGGSAIASGVAVSKVLHLEGEVNKIKSALASTNKAVVSLSNGISVLTSKVLDLKNIIDKQLLPIVNKQSCSISNIETVIEFQQKNNRLLEITREFSVNAGVTTPVSTYMLTNSELLSLINDMPITNDQKKLMSNNVQIVRQQSYSIMSIIKEEVLLYVVQLPLY

SEQ ID NO: 34 - protein, 222 aa, synthetic construct
GWYTSVITIELSNIKENKCNGTDAKVKLIKQELDKYKNAVTELQLLMQSTPATNNGGGPGGSAIASGVAVSKVLHLEGEVNKIKSALLSTNKAIVSLSNGVSVLTSKVLDLKNIIDKQLLPIVNKQSCSISNIETVIEFQQKNNRLLEITREFSVNAGVTTPVSTYMLTNSELLSLINDMPITNDQKKLMSNNVQIVRQQSYSIMSIIKEEVLAYVVQLPLY

SEQ ID NO: 35 - protein, 534 aa, synthetic construct
MELLILKANAITTILTAVTFCFASGQNITEEFYQSTCSAVSKGYLSALRTGWYTSVITIELSNIKKIKCNGTDAKIKLIKQELDKYKNAVTELQLLMQSTPATNNQARGSGSGRSLGFLLGVGSAIASGVAVSKVLHLEGEVNKIKSALLSTNKAVVSLSNGVSVLTSKVLDLKNYIDKQLLPIVNKQSCSIPNIETVIEFQQKNNRLLEITREFSVNAGVTTPVSTYMLTNSELLSLINDMPITNDQKKLMSNNVQIVRQQSYSIMSIIKEEVLAYVVQLPLYGVIDTPCWKLHTSPLCTTNTKEGSNICLTRTDRGWYCDNAGSVSFFPQAETCKVQSNRVFCDTMNSLTLPSEVNLCNVDIFNPKYDCKIMTSKTDVSSSVITSLGAIVSCYGKTKCTASNKNRGIIKTFSNGCDYVSNKGVDTVSVGNTLYYVNKQEGKSLYVKGEPIINFYDPLVFPSDQFDASISQVNEKINQSLAFIRKSDELLSAIGGYIPEAPRDGQAYVRKDGEWVLLSTFLGGIEGRHHHHHH

SEQ ID NO: 36 - protein, 225 aa, synthetic construct
QVTLRESGPALVKPTQTLTLTCTFSGFSLSTAGMSVGWIRQPPGKALEWLADIWWDDKKHYNPSLKDRLTISKDTSKNQVVLKVTNMDPADTATYYCARDMIFNFYFDVWGQGTTVTVSSASTKGPSVFPLAPSSKSTSGGTAALGCLVKDYFPEPVTVSWNSGALTSGVHTFPAVLQSSGLYSLSSVVTVPSSSLGTQTYICNVNHKPSNTKVDKKVEPKSCDK

SEQ ID NO: 37 - protein, 213 aa, synthetic construct
DIQMTQSPSTLSASVGDRVTITCSASSRVGYMHWYQQKPGKAPKLLIYDTSKLASGVPSRFSGSGSGTEFTLTISSLQPDDFATYYCFQGSGYPFTFGGGTKVEIKRTVAAPSVFIFPPSDEQLKSGTASVVCLLNNFYPREAKVQWKVDNALQSGNSQESVTEQDSKDSTYSLSSTLTLSKADYEKHKVYACEVTHQGLSSPVTKSFNRGEC

SEQ ID NO: 38 - protein, 231 aa, synthetic construct
QVQLVQSGAEVKKPGSSVMVSCQASGGPLRNYIINWLRQAPGQGPEWMGGIIPVLGTVHYAPKFQGRVTITADESTDTAYIHLISLRSEDTAMYYCATETALVVSTTYLPHYFDNWGQGTLVTVSSASTKGPSVFPLAPSSKSTSGGTAALGCLVKDYFPEPVTVSWNSGALTSGVHTFPAVLQSSGLYSLSSVVTVPSSSLGTQTYICNVNHKPSNTKVDKKVEPKSCDK

SEQ ID NO: 39 - protein, 214 aa, synthetic construct
DIQMTQSPSSLSAAVGDRVTITCQASQDIVNYLNWYQQKPGKAPKLLIYVASNLETGVPSRFSGSGSGTDFSLTISSLQPEDVATYYCQQYDNLPLTFGGGTKVEIKRTVAAPSVFIFPPSDEQLKSGTASVVCLLNNFYPREAKVQWKVDNALQSGNSQESVTEQDSKDSTYSLSSTLTLSKADYEKHKVYACEVTHQGLSSPVTKSFNRGEC

SEQ ID NO: 40 - protein, 225 aa, synthetic construct
EVQLVESGGGLVQPRRSLRLSCAASGFTFDDYTIHWVRQAPGKGLEWVSGITWNSGYIGYADSVKGRFTISRDNARNSLYLQMNSLRAEDTALYYCVRDAYVSGSDYYYYGLDVWGRGTLVTVSSASTKGPSVFPLAPSSKSTSGGTAALGCLVKDYFPEPVTVSWNSGALTSGVHTFPAVLQSSGLYSLSSVVTVPSSSLGTQTYICNVNHKPSNTKVDKKVEP

SEQ ID NO: 41 - protein, 214 aa, synthetic construct
EIVMTSSPATLSVSPGERVTLFCRASQSVISNLAWYQQKSGQAPRLLIYGASTRATGIPSRFSGSGSGTEFTLTISSLQSEDFAVYFCQQYNNWPLTFGGGTQVNVQRTVAAPSVFIFPPSDEQLKSGTASVVCLLNNFYPREAKVQWKVDNALQSGNSQESVTEQDSKDSTYSLSSTLTLSKADYEKHKVYACEVTHQGLSSPVTKSFNRGEC

SEQ ID NO: 42 - protein, 330 aa, synthetic construct [sequence omitted]

SEQ ID NO: 43 - protein, 107 aa, synthetic construct [sequence omitted]

SEQ ID NO: 44 - protein, 530 aa, synthetic construct; identical to SEQ ID NO: 11

SEQ ID NO: 45 - protein, 293 aa, synthetic construct
MDAMKRGLCCVLLLCGAVFVSAGGGSGGGWYTSVITIELSNIKENKCNGTDAKVKLLKQELDKYKNAVTELQLLMQSTPATNNGGGPGGSAIASGVAVSKVLHLEGEVNKIKSALLSTNKAVVSLSNGVSVLTSKVLDLKNYIDKQLLPIVNKQSCSISNIETVIEFQQKNNRLLEITREFSVNAGVTTPVSTYMLTNSELLSLINDMPITNDQKKLMSNNVQIVRQQSYSIMSIIKEEMLAYVVQLPLYGGGSGGGYIPEAPRDGQAYVRKDGEWVLLSTFLGSHHHHHHHH

SEQ ID NO: 46 - protein, 293 aa, synthetic construct
MDAMKRGLCCVLLLCGAVFVSAGGGSGGGWYTSVITIELSNIKENKCNGTDAKVKLLKQELDKYKNAVTELQLLMQSTPATNNGGGPGGSAIASGVAVSKVLHLEGEVNKIKSALLSTNKAVVSLSNGVSVLTSKVLDLKNYIDKQLLPIVNKQSCSISNIETVIEFQQKNNRLLEITREFSVNAGVTTPVSTYMLTNSELLSLINDMPITNDQKKLMSNNVQIVRQQSYSIMSIIKEEVLLYVVQLPLYGGGSGGGYIPEAPRDGQAYVRKDGEWVLLSTFLGSHHHHHHHH